European Patent Application EP 4 467 571 A1, published November 27, 2024. Title: ANTI-CD3/CD20 BISPECIFIC ANTIBODY AND USE THEREOF. Applicant: Shanghai Junshi Biosciences Co., Ltd. Application CN. The sequence listing filed with the application follows.

SEQUENCE LISTING (25 sequences)

SEQ ID NO: 1 - protein, 5 aa, synthetic construct
  REGION 1..5: note = CD20 HCDR1
YSWIN

SEQ ID NO: 2 - protein, 17 aa, synthetic construct
  REGION 1..17: note = CD20 HCDR2
RIFPGDGDTDYNGKFKG

SEQ ID NO: 3 - protein, 10 aa, synthetic construct
  REGION 1..10: note = CD20 HCDR3
NVFDGYWLVY

SEQ ID NO: 4 - protein, 16 aa, synthetic construct
  REGION 1..16: note = CD20 LCDR1
RSSKSLLHSNGITYLY

SEQ ID NO: 5 - protein, 7 aa, synthetic construct
  REGION 1..7: note = CD20 LCDR2
QMSNLVS

SEQ ID NO: 6 - protein, 9 aa, synthetic construct
  REGION 1..9: note = CD20 LCDR3
AQNLELPYT

SEQ ID NO: 7 - protein, 119 aa, synthetic construct
  REGION 1..119: note = CD20 VH
QVQLVQSGAEVKKPGSSVKVSCKASGYAFSYSWINWVRQAPGQGLEWMGRIFPGDGDTDYNGKFKGRVTITADKSTSTAYMELSSLRSEDTAVYYCARNVFDGYWLVYWGQGTLVTVSS

SEQ ID NO: 8 - protein, 112 aa, synthetic construct
  REGION 1..112: note = CD20 VL
DIVMTQTPLSLPVTPGEPASISCRSSKSLLHSNGITYLYWYLQKPGQSPQLLIYQMSNLVSGVPDRFSGSGSGTDFTLKISRVEAEDVGVYYCAQNLELPYTFGGGTKVEIK

SEQ ID NO: 9 - protein, 5 aa, synthetic construct
  REGION 1..5: note = JSCD3 HCDR1
TYAMN

SEQ ID NO: 10 - protein, 19 aa, synthetic construct
  REGION 1..19: note = JSCD3 HCDR2
RIRSKYNNYATYYADSVKD

SEQ ID NO: 11 - protein, 14 aa, synthetic construct
  REGION 1..14: note = JSCD3 HCDR3
HGNFGNSYVSWFAY

SEQ ID NO: 12 - protein, 14 aa, synthetic construct
  REGION 1..14: note = unknown
RSSTGAVTTSNYAN

SEQ ID NO: 13 - protein, 7 aa, synthetic construct
  REGION 1..7: note = JSCD3 LCDR2
GTNKRAP

SEQ ID NO: 14 - protein, 9 aa, synthetic construct
  REGION 1..9: note = JSCD3 LCDR3
ALWYSNLWV

SEQ ID NO: 15 - protein, 125 aa, synthetic construct
  REGION 1..125: note = JSCD3 VH
EVQLVESGGGLVQPGGSLKLSCAASGFTFSTYAMNWVRQAPGKCLEWVGRIRSKYNNYATYYADSVKDRFTISRDDSKNSLYLQMNSLKTEDTAVYYCVRHGNFGNSYVSWFAYWGQGTLVTVSS

SEQ ID NO: 16 - protein, 109 aa, synthetic construct
  REGION 1..109: note = JSCD3 VL
QAVVTQEPSLTVSPGGTVTLTCRSSTGAVTTSNYANWVQQKPGQAPRGLIGGTNKRAPGTPARFSGSLLGGKAALTLSGVQPEDEAEYYCALWYSNLWVFGCGTKLTVL

SEQ ID NO: 17 - protein, 446 aa, synthetic construct
  REGION 1..446: note = CD20 HC
QVQLVQSGAEVKKPGSSVKVSCKASGYAFSYSWINWVRQAPGQGLEWMGRIFPGDGDTDYNGKFKGRVTITADKSTSTAYMELSSLRSEDTAVYYCARNVFDGYWLVYWGQGTLVTVSSASTKGPSVFPLAPCSRSTSESTAALGCLVKDYFPEPVTVSWNSGALTSGVHTFPAVLQSSGLYSLSSVVTVPSSSLGTKTYTCNVDHKPSNTKVDKRVESKYGPPCPPCPAPEFLGGPSVFLFPPKPKDTLMISRTPEVTCVVVDVSQEDPEVQFNWYVDGVEVHNAKTKPREEQFNSTYRVVSVLTVLHQDWLNGKEYKCKVSNKGLPSSIEKTISKAKGQPREPQVYTLPPCQEEMTKNQVSLWCLVKGFYPSDIAVEWESNGQPENNYKTTPPVLDSDGSFFLYSRLTVDKSRWQEGNVFSCSVMHEALHNHYTQKSLSLSLGK

SEQ ID NO: 18 - protein, 219 aa, synthetic construct
  REGION 1..219: note = CD20 LC
DIVMTQTPLSLPVTPGEPASISCRSSKSLLHSNGITYLYWYLQKPGQSPQLLIYQMSNLVSGVPDRFSGSGSGTDFTLKISRVEAEDVGVYYCAQNLELPYTFGGGTKVEIKRTVAAPSVFIFPPSDEQLKSGTASVVCLLNNFYPREAKVQWKVDNALQSGNSQESVTEQDSKDSTYSLSSTLTLSKADYEKHKVYACEVTHQGLSSPVTKSFNRGEC

SEQ ID NO: 19 - protein, 722 aa, synthetic construct
  REGION 1..722: note = CD20 and CD3 mixed HC
QVQLVQSGAEVKKPGSSVKVSCKASGYAFSYSWINWVRQAPGQGLEWMGRIFPGDGDTDYNGKFKGRVTITADKSTSTAYMELSSLRSEDTAVYYCARNVFDGYWLVYWGQGTLVTVSSASTKGPSVFPLAPCSRSTSESTAALGCLVKDYFPEPVTVSWNSGALTSGVHTFPAVLQSSGLYSLSSVVTVPSSSLGTKTYTCNVDHKPSNTKVDKRVASGGGGSGGGGSQAVVTQEPSLTVSPGGTVTLTCRSSTGAVTTSNYANWVQQKPGQAPRGLIGGTNKRAPGTPARFSGSLLGGKAALTLSGVQPEDEAEYYCALWYSNLWVFGCGTKLTVLGGGGSGGGGSGGGGSGGGGSEVQLVESGGGLVQPGGSLKLSCAASGFTFSTYAMNWVRQAPGKCLEWVGRIRSKYNNYATYYADSVKDRFTISRDDSKNSLYLQMNSLKTEDTAVYYCVRHGNFGNSYVSWFAYWGQGTLVTVSSGGGGSGGGGSESKYGPPCPPCPAPEFLGGPSVFLFPPKPKDTLMISRTPEVTCVVVDVSQEDPEVQFNWYVDGVEVHNAKTKPREEQFNSTYRVVSVLTVLHQDWLNGKEYKCKVSNKGLPSSIEKTISKAKGQPREPQVYTLPPCQEEMTKNQVSLWCLVKGFYPSDIAVEWESNGQPENNYKTTPPVLDSDGSFFLYSRLTVDKSRWQEGNVFSCSVMHEALHNHYTQKSLSLSLGK

SEQ ID NO: 20 - protein, 493 aa, synthetic construct
  REGION 1..493: note = CD3 HLFc
QAVVTQEPSLTVSPGGTVTLTCRSSTGAVTTSNYANWVQQKPGQAPRGLIGGTNKRAPGTPARFSGSLLGGKAALTLSGVQPEDEAEYYCALWYSNLWVFGCGTKLTVLGGGGSGGGGSGGGGSGGGGSEVQLVESGGGLVQPGGSLKLSCAASGFTFSTYAMNWVRQAPGKCLEWVGRIRSKYNNYATYYADSVKDRFTISRDDSKNSLYLQMNSLKTEDTAVYYCVRHGNFGNSYVSWFAYWGQGTLVTVSSGGGGSGGGGSESKYGPPCPPCPAPEFLGGPSVFLFPPKPKDTLMISRTPEVTCVVVDVSQEDPEVQFNWYVDGVEVHNAKTKPREEQFNSTYRVVSVLTVLHQDWLNGKEYKCKVSNKGLPSSIEKTISKAKGQPREPQVCTLPPSQEEMTKNQVSLSCAVKGFYPSDIAVEWESNGQPENNYKTTPPVLDSDGSFFLVSRLTVDKSRWQEGNVFSCSVMHEALHNRFTQKSLSLSLGK

SEQ ID NO: 21 - protein, 452 aa, synthetic construct
  REGION 1..452: note = JSCD3 HC
EVQLVESGGGLVQPGGSLKLSCAASGFTFSTYAMNWVRQAPGKGLEWVGRIRSKYNNYATYYADSVKDRFTISRDDSKNSLYLQMNSLKTEDTAVYYCVRHGNFGNSYVSWFAYWGQGTLVTVSSASTKGPSVFPLAPCSRSTSESTAALGCLVKDYFPEPVTVSWNSGALTSGVHTFPAVLQSSGLYSLSSVVTVPSSSLGTKTYTCNVDHKPSNTKVDKRVESKYGPPCPPCPAPEFLGGPSVFLFPPKPKDTLMISRTPEVTCVVVDVSQEDPEVQFNWYVDGVEVHNAKTKPREEQFNSTYRVVSVLTVLHQDWLNGKEYKCKVSNKGLPSSIEKTISKAKGQPREPQVYTLPPSQEEMTKNQVSLTCLVKGFYPSDIAVEWESNGQPENNYKTTPPVLDSDGSFFLYSRLTVDKSRWQEGNVFSCSVMHEALHNHYTQKSLSLSLGK

SEQ ID NO: 22 - protein, 216 aa, synthetic construct
  REGION 1..216: note = JSCD3 LC
QAVVTQEPSLTVSPGGTVTLTCRSSTGAVTTSNYANWVQQKPGQAPRGLIGGTNKRAPGTPARFSGSLLGGKAALTLSGVQPEDEAEYYCALWYSNLWVFGGGTKLTVLRTVAAPSVFIFPPSDEQLKSGTASVVCLLNNFYPREAKVQWKVDNALQSGNSQESVTEQDSKDSTYSLSSTLTLSKADYEKHKVYACEVTHQGLSSPVTKSFNRGEC

SEQ ID NO: 23 - protein, 446 aa, synthetic construct
  REGION 1..446: note = CD20 HC
QVQLVQSGAEVKKPGSSVKVSCKASGYAFSYSWINWVRQAPGQGLEWMGRIFPGDGDTDYNGKFKGRVTITADKSTSTAYMELSSLRSEDTAVYYCARNVFDGYWLVYWGQGTLVTVSSASTKGPSVFPLAPCSRSTSESTAALGCLVKDYFPEPVTVSWNSGALTSGVHTFPAVLQSSGLYSLSSVVTVPSSSLGTKTYTCNVDHKPSNTKVDKRVESKYGPPCPPCPAPEFLGGPSVFLFPPKPKDTLMISRTPEVTCVVVDVSQEDPEVQFNWYVDGVEVHNAKTKPREEQFNSTYRVVSVLTVLHQDWLNGKEYKCKVSNKGLPSSIEKTISKAKGQPREPQVCTLPPSQEEMTKNQVSLSCAVKGFYPSDIAVEWESNGQPENNYKTTPPVLDSDGSFFLVSRLTVDKSRWQEGNVFSCSVMHEALHNRFTQKSLSLSLGK

SEQ ID NO: 24 - protein, 452 aa, synthetic construct
  REGION 1..452: note = heavy chain
EVQLVESGGGLVQPKGSLKLSCAASGFTFNTYAMNWVRQAPGKGLEWVARIRSKYNNYATYYADSVKDRFTISRDDSQSILYLQMNNLKTEDTAMYYCVRHGNFGNSYVSWFAYWGQGTLVTVSAASTKGPSVFPLAPCSRSTSESTAALGCLVKDYFPEPVTVSWNSGALTSGVHTFPAVLQSSGLYSLSSVVTVPSSSLGTKTYTCNVDHKPSNTKVDKRVESKYGPPCPPCPAPEFLGGPSVFLFPPKPKDTLMISRTPEVTCVVVDVSQEDPEVQFNWYVDGVEVHNAKTKPREEQFNSTYRVVSVLTVLHQDWLNGKEYKCKVSNKGLPSSIEKTISKAKGQPREPQVYTLPPSQEEMTKNQVSLTCLVKGFYPSDIAVEWESNGQPENNYKTTPPVLDSDGSFFLYSRLTVDKSRWQEGNVFSCSVMHEALHNHYTQKSLSLSLGK

SEQ ID NO: 25 - protein, 216 aa, synthetic construct
  REGION 1..216: note = light chain
QAVVTQESALTTSPGETVTLTCRSSTGAVTTSNYANWVQEKPDHLFTGLIGGTNKRAPGVPARFSGSLIGDKAALTITGAQTEDEAIYFCALWYSNLWVFGGGTKLTVLRTVAAPSVFIFPPSDEQLKSGTASVVCLLNNFYPREAKVQWKVDNALQSGNSQESVTEQDSKDSTYSLSSTLTLSKADYEKHKVYACEVTHQGLSSPVTKSFNRGEC